European Patent Application EP 4 741 426 A1, published May 13, 2026. Title: 一种抗体和IL-2的复合体及其应用. Applicant: 北京志道生物科技有限公司. Application CN. The sequence listing filed with the application follows.

SEQUENCE LISTING (25 sequences)

SEQ ID NO: 1 - protein, 24 aa, unidentified
NNYKNPKLTRMLTFKFYMPKKATE

SEQ ID NO: 2 - protein, 20 aa, unidentified
LKHLQCLEEELKPLEEVLNL

SEQ ID NO: 3 - protein, 9 aa, unidentified
AQSKNFHLR

SEQ ID NO: 4 - protein, 16 aa, unidentified
PRDLISNINVIVLELK

SEQ ID NO: 5 - protein, 16 aa, unidentified
GSETTFMCEYADETAT

SEQ ID NO: 6 - protein, 20 aa, unidentified
IVEFLNRWITFCQSIISTLT

SEQ ID NO: 7 - protein, 133 aa, unidentified [sequence omitted]

SEQ ID NO: 8 - protein, 19 aa, unidentified
QSMHIDATLYTESDVHPSC

SEQ ID NO: 9 - protein, 18 aa, unidentified
KVTAMKCFLLELQVISLE

SEQ ID NO: 10 - protein, 5 aa, unidentified
SGDAS

SEQ ID NO: 11 - protein, 16 aa, unidentified
IHDTVENLIILANNSL

SEQ ID NO: 12 - protein, 21 aa, unidentified
SSNGNVTESGCKECEELEEKN

SEQ ID NO: 13 - protein, 114 aa, unidentified
NWVNVISDLKKIEDLIQSMHIDATLYTESDVHPSCKVTAMKCFLLELQVISLESGDASIHDTVENLIILANNSLSSNGNVTESGCKECEELEEKNIKEFLQSFVHIVQMFINTS

SEQ ID NO: 14 - protein, 127 aa, unidentified
APTSSSTKKTQLQLEHLLLDLQMILNGIQSMHIDATLYTESDVHPSCKVTAMKCFLLELQVISLESGDASIHDTVENLIILANNSLSSNGNVTESGCKECEELEEKNIVEFLNRFITFAQSIISTLT

SEQ ID NO: 15 - protein, 127 aa, unidentified
APTSSSTKKTQLQLEHLLLDLQMILNGIQSMHIDATLYTESDVHPSCKVTAMKCFLLELQVISLESGDASIHDTVEDLIILANNSLSSNGNVTESGCKECEELEEKNIVEFLNRFITFAQSIISTLT

SEQ ID NO: 16 - protein, 127 aa, unidentified
APTSSSTKKTQLQLEHLLLDLQMILNGIQSMHIDATLYTESDVHPSCKVTAMKCFLLELQVISLESGDASIHDTVQNLIILANNSLSSNGNVTESGCKECEELEEKNIVEFLNRFITFAQSIISTLT

SEQ ID NO: 17 - protein, 127 aa, unidentified
APTSSSTKKTQLQLEHLLLDLQMILNGIQSMHIDATLYTESDVHPSCKVTAMKCFLLELQVISLESGDASIHDTVENLITLANNSLSSNGNVTESGCKECEELEEKNIVEFLNRFITFAQSIISTLT

SEQ ID NO: 18 - protein, 127 aa, unidentified
APTSSSTKKTQLQLEHLLLDLQMILNGIQSMHIDATLYTESDVHPSCKVTAMKCFLLELQVISLESGDASIHDTVENLIITANNSLSSNGNVTESGCKECEELEEKNIVEFLNRFITFAQSIISTLT

SEQ ID NO: 19 - protein, 65 aa, unidentified
ITCPPPMSVEHADIWVKSYSLYSRERYICNSGFKRKAGTSSLTECVLNKATNVAHWTTPSLKCIR

SEQ ID NO: 20 - protein, 214 aa, unidentified
EIVLTQSPATLSLSPGERATLSCRASQSVSSYLAWYQQKPGQAPRLLIYDASKRATGIPARFSGSGSGTDFTLTISSLEPEDFAVYYCDQRNNWPLTFGGGTKVEIKRTVAAPSVFIFPPSDEQLKSGTASVVCLLNNFYPREAKVQWKVDNALQSGNSQESVTEQDSKDSTYSLSSTLTLSKADYEKHKVYACEVTHQGLSSPVTKSFNRGEC

SEQ ID NO: 21 - protein, 523 aa, unidentified
QVQLVQSGAEVKKPGASVKVSCKASGYTFTAQYMHWVRQAPGQGLEWMGIINPSGGETGYAQKFQGRVTMTRDTSTSTVYMELSSLRSEDTAVYYCAKEGVADGYGLVDVWGQGTMVTVSSASTKGPSVFPLAPCSRSTSESTAALGCLVKDYFPEPVTVSWNSGALTSGVHTFPAVLQSSGLYSLSSVVTVPSSSLGTKTYTCNVDHKPSNTKVDKRVESKYGPPCPPCPAPEFLGGPSVFLFPPKPKDTLMISRTPEVTCVVVDVSQEDPEVQFNWYVDGVEVHNAKTKPREEQFNSTYRVVSVLTVLHQDWLNGKEYKCKVSNKGLPSSIEKTISKAKGQPREPQVYTLPPSQEEMTKNQVSLTCLVKGFYPSDIAVEWESNGQPENNYKTTPPVLDSDGSFFLYSRLTVDKSRWQEGNVFSCSVMHEALHNHYTQKSLSLSLGKGGGGSGGGGSITCPPPMSVEHADIWVKSYSLYSRERYICNSGFKRKAGTSSLTECVLNKATNVAHWTTPSLKCIR

SEQ ID NO: 22 - protein, 293 aa, unidentified
ITCPPPMSVEHADIWVKSYSLYSRERYICNSGFKRKAGTSSLTECVLNKATNVAHWTTPSLKCIRESKYGPPCPPCPAPEFLGGPSVFLFPPKPKDTLMISRTPEVTCVVVDVSQEDPEVQFNWYVDGVEVHNAKTKPREEQFNSTYRVVSVLTVLHQDWLNGKEYKCKVSNKGLPSSIEKTISKAKGQPREPQVYTLPPSQEEMTKNQVSLTCLVKGFYPSDIAVEWESNGQPENNYKTTPPVLDSDGSFFLYSRLTVDKSRWQEGNVFSCSVMHEALHNHYTQKSLSLSLG

SEQ ID NO: 23 - protein, 126 aa, unidentified
APTSSSTKKTQLQLEHLLLDLQMILNGIQSMHIDATLYTESDVHPSCKVTAMKCFLLELQVISLESGDASIHDTVENLIILANNSLSSNGNVTESGCKECEELEEKNIVEFLNRFITFAQSIISTL

SEQ ID NO: 24 - protein, 125 aa, unidentified
APTSSSTKKTQLQLEHLLLDLQMILNGIQSMHIDATLYTESDVHPSCKVTAMKCFLLELQVISLESGDASIHDTVENLIILANNSLSSNGNVTESGCKECEELEEKNIVEFLNRFITFAQSIIST

SEQ ID NO: 25 - protein, 124 aa, unidentified
APTSSSTKKTQLQLEHLLLDLQMILNGIQSMHIDATLYTESDVHPSCKVTAMKCFLLELQVISLESGDASIHDTVENLIILANNSLSSNGNVTESGCKECEELEEKNIVEFLNRFITFAQSIIS